European Patent Specification EP 3 469 080 B1, published July 15, 2026. Title: OPTIMIZED CLN1 GENES AND EXPRESSION CASSETTES AND THEIR USE. Applicant: The University of North Carolina at Chapel Hill Gray, Steven. The sequence listing filed with the application follows.

SEQUENCE LISTING (7 sequences)

SEQ ID NO: 1 - DNA, 924 bp, Artificial
  Human codon-optimized CLN1 open reading frame
atggcttctccggggtgtctgtggctgctggcagtggcactccttccctggacttgcgccagccgggctctgcagcacctcgaccctccagcccctcttccactggtgatttggcacggaatgggtgattcctgctgtaatcccctgtcaatgggagccatcaagaagatggtggagaagaagatccctggaatctacgtgctgtcactggagattggaaagaccctgatggaggacgtcgagaactccttcttcctcaatgtcaactctcaagtgaccaccgtctgccaggccctggccaaggacccgaagctgcagcaggggtataatgctatggggttcagccagggaggacagttccttcgggctgtggcccaacgctgccctagcccacccatgatcaacctgatctcagtgggtggccagcatcagggcgtgttcggacttccccggtgtcccggggaatcctctcatatctgcgacttcatccgcaaaactctcaatgcaggcgcttattcaaaggtcgtccaagagaggctggtgcaagccgagtactggcacgatcccattaaggaggacgtgtacagaaatcactcaatctttctggccgacattaaccaggagaggggaattaacgaatcatataagaagaatctcatggccctcaaaaagttcgtcatggtgaagttccttaacgatagcattgtggacccagtggacagcgaatggttcggattttaccgctcaggccaggcaaaagaaaccatccctctccaagagacttctctttacacccaagacagacttgggcttaaggaaatggataacgctggtcagctggtgttcctcgccaccgaaggtgaccatctgcagctcagcgaagagtggttctacgctcatatcatcccgtttcttggttgataa

SEQ ID NO: 2 - DNA, 306 bp, Chicken beta-actin promoter
tacgtattagtcatcgctattaccatggtcgaggtgagccccacgttctgcttcactctccccatctcccccccctccccacccccaattttgtatttatttattttttaattattttgtgcagcgatgggggcggggggggggggggggcgcgcgccaggcggggcggggcggggcgaggggcggggcggggcgaggcggagaggtgcggcggcagccaatcagagcggcgcgctccgaaagtttccttttatggcgaggcggcggcggcggcggccctataaaaagcgaagcgcgcggcgggcg

SEQ ID NO: 3 - DNA, 137 bp, Chicken beta-actin exon 1 and intron 1
ggagtcgctgcgacgctgccttcgccccgtgccccgctccgccgccgcctcgcgccgcccgccccggctctgactgaccgcgttactcccacaggtgagcgggcgggacggcccttctcctccgggctgtaattagc

SEQ ID NO: 4 - DNA, 256 bp, Cytomegalovirus enhancer
tacataacttacggtaaatggcccgcctggctgaccgcccaacgacccccgcccattgacgtcaatagtaacgccaatagggactttccattgacgtcaatgggtggagtatttacggtaaactgcccacttggcagtacatcaagtgtatcatatgccaagtacgccccctattgacgtcaatgacggtaaatggcccgcctggcattgtgcccagtacatgaccttatgggactttcctacttggcagtacatc

SEQ ID NO: 5 - DNA, 92 bp, Artificial
  Hybrid/modified MVM intron
aagaggtaagggtttaagggatggttggttggtggggtattaatgtttaattacctggagcacctgcctgaaatcactttttttcaggttgg

SEQ ID NO: 6 - DNA, 254 bp, Bovine growth hormone polyadenylation signal
ctcgactgtgccttctagttgccagccatctgttgtttgcccctcccccgtgccttccttgaccctggaaggtgccactcccactgtcctttcctaataaaatgaggaaattgcatcgcattgtctgagtaggtgtcattctattctggggggtggggtggggcaggacagcaagggggaggattgggaagacaacagcaggcatgctggggatgcggtgggctctatggcttctgaggcggaaagaaccagct

SEQ ID NO: 7 - DNA, 2302 bp, Artificial
  CLN1 expression cassette
ctgcgcgctcgctcgctcactgaggccgcccgggcaaagcccgggcgtcgggcgacctttggtcgcccggcctcagtgagcgagcgagcgcgcagagagggagtggggttcggtacccgttacataacttacggtaaatggcccgcctggctgaccgcccaacgacccccgcccattgacgtcaatagtaacgccaatagggactttccattgacgtcaatgggtggagtatttacggtaaactgcccacttggcagtacatcaagtgtatcatatgccaagtacgccccctattgacgtcaatgacggtaaatggcccgcctggcattgtgcccagtacatgaccttatgggactttcctacttggcagtacatctacgtattagtcatcgctattaccatggtcgaggtgagccccacgttctgcttcactctccccatctcccccccctccccacccccaattttgtatttatttattttttaattattttgtgcagcgatgggggcggggggggggggggggcgcgcgccaggcggggcggggcggggcgaggggcggggcggggcgaggcggagaggtgcggcggcagccaatcagagcggcgcgctccgaaagtttccttttatggcgaggcggcggcggcggcggccctataaaaagcgaagcgcgcggcgggcgggagtcgctgcgacgctgccttcgccccgtgccccgctccgccgccgcctcgcgccgcccgccccggctctgactgaccgcgttactcccacaggtgagcgggcgggacggcccttctcctccgggctgtaattagctgagcaagaggtaagggtttaagggatggttggttggtggggtattaatgtttaattacctggagcacctgcctgaaatcactttttttcaggttggaccggtcgccaccatggcttctccggggtgtctgtggctgctggcagtggcactccttccctggacttgcgccagccgggctctgcagcacctcgaccctccagcccctcttccactggtgatttggcacggaatgggtgattcctgctgtaatcccctgtcaatgggagccatcaagaagatggtggagaagaagatccctggaatctacgtgctgtcactggagattggaaagaccctgatggaggacgtcgagaactccttcttcctcaatgtcaactctcaagtgaccaccgtctgccaggccctggccaaggacccgaagctgcagcaggggtataatgctatggggttcagccagggaggacagttccttcgggctgtggcccaacgctgccctagcccacccatgatcaacctgatctcagtgggtggccagcatcagggcgtgttcggacttccccggtgtcccggggaatcctctcatatctgcgacttcatccgcaaaactctcaatgcaggcgcttattcaaaggtcgtccaagagaggctggtgcaagccgagtactggcacgatcccattaaggaggacgtgtacagaaatcactcaatctttctggccgacattaaccaggagaggggaattaacgaatcatataagaagaatctcatggccctcaaaaagttcgtcatggtgaagttccttaacgatagcattgtggacccagtggacagcgaatggttcggattttaccgctcaggccaggcaaaagaaaccatccctctccaagagacttctctttacacccaagacagacttgggcttaaggaaatggataacgctggtcagctggtgttcctcgccaccgaaggtgaccatctgcagctcagcgaagagtggttctacgctcatatcatcccgtttcttggttgataagcggccgcggggatccctcgactgtgccttctagttgccagccatctgttgtttgcccctcccccgtgccttccttgaccctggaaggtgccactcccactgtcctttcctaataaaatgaggaaattgcatcgcattgtctgagtaggtgtcattctattctggggggtggggtggggcaggacagcaagggggaggattgggaagacaacagcaggcatgctggggatgcggtgggctctatggcttctgaggcggaaagaaccagctttggacgcgtaggaacccctagtgatggagttggccactccctctctgcgcgctcgctcgctcactgaggccgggcgaccaaaggtcgcccgacgcccgggctttgcccgggcggcctcagtgagcgagcgagcgcgcagctggcgtaatagcgaagaggcccgcaccgatcgcccttc